European Patent Specification EP 3 368 562 B1, published December 17, 2025. Title: MONOCLONAL ANTIBODY NEUTRALIZING HUMAN RESPIRATORY SYNCYTIAL VIRUS. Applicant: Vora, Kalpit A. Cox, Kara S. Tang, Aimin Chen, Zhifeng DiStefano, Daniel Zhang, Lan Su, Hua-Poo. Application US 62/367,359. The sequence listing filed with the application follows.

SEQUENCE LISTING (22 sequences)

SEQ ID NO: 1 - protein, 5 aa, Homo sapiens
DSAMS

SEQ ID NO: 2 - protein, 19 aa, Homo sapiens
FIKSKTYGGTKEYAASVKG

SEQ ID NO: 3 - protein, 16 aa, Homo sapiens
GAPYGGNSDYYYGLDV

SEQ ID NO: 4 - protein, 11 aa, Homo sapiens
RTSQDVRGALA

SEQ ID NO: 5 - protein, 7 aa, Homo sapiens
DASSLET

SEQ ID NO: 6 - protein, 9 aa, Homo sapiens
QQFLDFPFT

SEQ ID NO: 7 - protein, 127 aa, Artificial Sequence
  RB1 heavy chain with amino acid substitution
EVQLVESGGGLVRPGRSLRLSCTVSGFSFDDSAMSWVRQAPGKGLEWISFIKSKTYGGTKEYAASVKGRFTISRDDSKNIAYLQMNSLKTEDTAVYYCTRGAPYGGNSDYYYGLDVWGQGTTVTVSS

SEQ ID NO: 8 - protein, 109 aa, Homo sapiens
DIQMTQSPSSLSASVGDRVTITCRTSQDVRGALAWYQQKPGKAPKLLIFDASSLETGVPSRFSGSGSGTVFTLTISSLQPEDFAAYYCQQFLDFPFTFGQGTRLEIKRT

SEQ ID NO: 9 - protein, 127 aa, Homo sapiens
EVQLVESGGGLVRPGRSLRLSCTVSGFSFDDSAMSWVRQAPGKGLEWISFIKSKTYGGTKEYAASVKGRFTISRDDSKNIAYLQMNSLKTEDTAVYYCTRGAPYGGNSDYYYGLDVWGQGTTVIVSS

SEQ ID NO: 10 - protein, 19 aa, Artificial Sequence
  Leader sequence
MGWSCIILFLVATATGVHS

SEQ ID NO: 11 - protein, 146 aa, Artificial Sequence
  RB1 VH amino acid substituted with leader
MGWSCIILFLVATATGVHSEVQLVESGGGLVRPGRSLRLSCTVSGFSFDDSAMSWVRQAPGKGLEWISFIKSKTYGGTKEYAASVKGRFTISRDDSKNIAYLQMNSLKTEDTAVYYCTRGAPYGGNSDYYYGLDVWGQGTTVTVSS

SEQ ID NO: 12 - protein, 128 aa, Artificial Sequence
  RB1 VL and leader
MGWSCIILFLVATATGVHSDIQMTQSPSSLSASVGDRVTITCRTSQDVRGALAWYQQKPGKAPKLLIFDASSLETGVPSRFSGSGSGTVFTLTISSLQPEDFAAYYCQQFLDFPFTFGQGTRLEIKRT

SEQ ID NO: 13 - protein, 330 aa, Homo sapiens [sequence omitted]

SEQ ID NO: 14 - protein, 105 aa, Homo sapiens [sequence omitted]

SEQ ID NO: 15 - DNA, 381 bp, Artificial Sequence
  RB1 with amino acid substitution
gaggtgcagctggtggagtctgggggaggcttggtacggccagggcggtccctgagactctcctgcacagtttctggattcagctttgacgactctgctatgagctgggtccgccaggctccagggaaggggctggaatggataagtttcattaaaagtaaaacttatggtgggacaaaagaatacgccgcgtctgtgaaaggcaggttcaccatctcaagagatgattccaaaaacatcgcctatctgcaaatgaacagcctgaaaaccgaggacacagccgtgtattattgtactagaggggcgccttacggcggtaactccgattactactacggtttggacgtctggggccaagggaccacggtcactgtctcctca

SEQ ID NO: 16 - DNA, 327 bp, Homo sapiens
gacatccagatgacccagtctccatcctccctgtctgcatctgtaggagacagagtcaccatcacttgccggacaagtcaggacgttagaggtgctttagcctggtatcaacagaaaccagggaaagctcctaaactcctgatctttgatgcctccagtttggagactggggtcccatcaaggttcagcggcagtggatctgggacagttttcactctcaccatcagcagcctgcagcctgaagattttgcagcttattactgtcagcagtttcttgatttccctttcaccttcggccaggggacacgactggaaatcaaacgtacg

SEQ ID NO: 17 - DNA, 381 bp, Artificial Sequence
  RB1 VH codon optimized
gaggtgcagctggtcgagagcgggggggggctggtgcggcctggcaggtctctgagactgagctgcaccgtgagcggcttctcctttgacgattctgccatgagctgggtgcggcaggctccaggcaagggactggagtggatctccttcatcaagtctaagacctacggcggcacaaaggagtacgccgcttccgtgaagggccggtttaccatcagcagggacgattccaagaacatcgcctatctgcagatgaacagcctgaagaccgaggacacagccgtgtactattgcacaagaggagctccttacggaggcaacagcgactactattacggactggacgtgtggggacagggaaccacagtgaccgtgagctcc

SEQ ID NO: 18 - DNA, 327 bp, Artificial Sequence
  RB1 VL codon optimized
gacattcagatgactcagtccccttcaagtctgagcgcctccgtgggcgacagagtgaccatcacatgccggaccagccaggatgtgcggggcgccctggcttggtaccagcagaagccaggcaaggcccccaagctgctgatctttgacgctagctccctggagaccggcgtgccctccaggttttctggcagcggctccggcacagtgttcaccctgacaatctctagcctgcagcctgaggactttgccgcttactattgccagcagttcctggatttccccttcaccttcggccaaggcacacggctggagatcaagaggacc

SEQ ID NO: 19 - DNA, 57 bp, Artificial Sequence
  Leader sequence heavy chain
atgggttggtcctgtattatcctgttcctggtcgccactgctactggggtccactca

SEQ ID NO: 20 - DNA, 57 bp, Artificial Sequence
  Leader sequence light chain
atgggctggtcctgtattatcctgttcctggtggcaaccgcaactggtgtgcatagc

SEQ ID NO: 21 - DNA, 990 bp, Homo sapiens
gcctctacaaagggccctagcgtgttcccactggctccctcttccaagtctaccagcggaggaacagccgctctgggatgtctggtgaaggattacttcccagagcccgtgaccgtgtcctggaactctggcgccctgaccagcggagtgcacacatttccagctgtgctgcagtcctctggcctgtattccctgagctccgtggtgaccgtgccctctagctccctgggcacccagacatacatctgtaacgtgaatcacaagccaagcaatacaaaggtggacaagaaggtcgagcccaagtcctgtgataagacccacacatgccccccttgtcctgctccagagctgctgggaggacctagcgtgttcctgtttccacccaagcctaaggacaccctgatgatctctaggacccccgaggtgacatgcgtggtggtggacgtgagccacgaggatcctgaggtgaagtttaactggtacgtcgatggcgtggaggtgcacaatgccaagacaaagcccagagaggagcagtataactccacctaccgggtggtgtctgtgctgacagtgctgcaccaggactggctgaacggcaaggagtacaagtgcaaggtgtccaataaggccctgcccgctcctatcgagaagaccatctctaaggccaagggccagcctagggagccacaggtgtatacactgcctccatccagagacgagctgaccaagaaccaggtgtctctgacatgtctggtgaagggcttctacccttctgatatcgccgtggagtgggagagcaatggccagccagagaacaattataagaccacaccccctgtgctggacagcgatggctccttctttctgtacagcaagctgaccgtggataagtcccggtggcagcagggcaacgtgttcagctgttctgtgatgcacgaagccctgcacaatcactacactcagaagagcctgtccctgtcacctggtaaa

SEQ ID NO: 22 - DNA, 315 bp, Homo sapiens
gtggccgctccctccgtgtttatcttccccccttctgacgagcagctgaagtctggcacagctagcgtggtgtgcctgctgaacaatttctaccctcgggaggccaaggtgcagtggaaggtggataacgctctgcagtctggcaatagccaggagtccgtgaccgagcaggactctaaggatagcacatattccctgtcctctaccctgacactgtctaaggccgattacgagaagcacaaggtgtatgcttgtgaagtcacccaccaggggctgagttcaccagtcaccaagtcattcaatcggggcgagtgc